European Patent Specification EP 3 609 519 B1, published November 26, 2025. Title: Compositions and Methods for Treating Inflammation and Cancer. Applicant: University of Maryland Bromberg, Jonathan Piao, Wenji Xiong, Yanbao. The sequence listing filed with the application follows.

SEQUENCE LISTING (10 sequences)

SEQ ID NO: 1 - protein, 16 aa, Artificial Sequence
  Chemically Synthesized
RQIKIWFQNRRMKWKK

SEQ ID NO: 2 - protein, 12 aa, Artificial Sequence
  Chemically Synthesized
TGNIYIYNGPVL

SEQ ID NO: 3 - protein, 8 aa, Artificial Sequence
  Chemically Synthesized
PEEGAPGP

SEQ ID NO: 4 - protein, 28 aa, Artificial Sequence
  Chemically Synthesized
RQIKIWFQNRRMKWKKTGNIYIYNGPVL

SEQ ID NO: 5 - protein, 24 aa, Artificial Sequence
  Chemically Synthesized
RQIKIWFQNRRMKWKKPEEGAPGP

SEQ ID NO: 6 - protein, 12 aa, Artificial Sequence
  Chemically Synthesized
CMHIESLDSYTC

SEQ ID NO: 7 - protein, 12 aa, Artificial Sequence
  Chemically Synthesized
CMYIEALDKYAC

SEQ ID NO: 8 - protein, 29 aa, Artificial Sequence
  Chemically Synthesized
EAALAEALAEALAEALAEALAEALEALAA

SEQ ID NO: 9 - protein, 8 aa, Artificial Sequence
  Chemically Synthesized
GNAAAARR

SEQ ID NO: 10 - protein, 10 aa, Artificial Sequence
  Chemically Synthesized
CDPGYIGSRC